European Patent Specification EP 3 736 341 B1, published August 23, 2023. Title: ERROR SUPPRESSION IN SEQUENCED DNA FRAGMENTS USING REDUNDANT READS WITH UNIQUE MOLECULAR INDICES (UMIS). Applicant: Illumina, Inc. The sequence listing filed with the application follows.

SEQUENCE LISTING (3 sequences)

SEQ ID NO: 1 - DNA, 15 bp, Artificial Sequence
  Synthetic polynucleotide
  misc_feature (4)..(7): n is a, c, g, or t
  misc_feature (9)..(12): n is a, c, g, or t
ccannnnannnntgg

SEQ ID NO: 2 - DNA, 45 bp, Artificial Sequence
  Synthetic polynucleotide
  misc_feature (1)..(4): n is a, c, g, or t
nnnntgctcgcagatcggaagagcacacgtctgaactccagtcac

SEQ ID NO: 3 - DNA, 44 bp, Artificial Sequence
  Synthetic polynucleotide
  misc_feature (40)..(43): n is a, c, g, or t
cactctttccctacacgacgctcttccgatctgcgaccannnnt